European Patent Application EP 4 316 483 A1, published February 7, 2024. Title: COMPOSITIN FOR ENHANCING THE ACTIVITY OF LACTIC ACID BACTERIA. Applicant: SEOUL NATIONAL UNIVERSITY R&DB FOUNDATION. The sequence listing filed with the application follows.

SEQUENCE LISTING (22 sequences)

SEQ ID NO: 1 - DNA, 20 bp, Artificial Sequence
  CNMa_Forward primer
tgtgatccttgaggggatgt

SEQ ID NO: 2 - DNA, 20 bp, Artificial Sequence
  CNMa_Reverse primer
caacagcaggaacagaagca

SEQ ID NO: 3 - DNA, 21 bp, Artificial Sequence
  AstA_Forward primer
gaggtctcgtccctatccttc

SEQ ID NO: 4 - DNA, 20 bp, Artificial Sequence
  AstA_Reverse primer
gatctcgttgtcctggtcgt

SEQ ID NO: 5 - DNA, 20 bp, Artificial Sequence
  AstB_Forward primer
tttggtggccagtggtagtg

SEQ ID NO: 6 - DNA, 20 bp, Artificial Sequence
  AstB_Reverse primer
gtcgctctcgctaagttggt

SEQ ID NO: 7 - DNA, 19 bp, Artificial Sequence
  AstC_Forward primer
gcgcctatttgaggagtcc

SEQ ID NO: 8 - DNA, 19 bp, Artificial Sequence
  AstC_Reverse primer
cttgacgtttgctctcggg

SEQ ID NO: 9 - DNA, 19 bp, Artificial Sequence
  CCHa1_Forward primer
tcgtcgagaatcggaggat

SEQ ID NO: 10 - DNA, 16 bp, Artificial Sequence
  CCHa1_Reverse primer
actggcgcaattgata

SEQ ID NO: 11 - DNA, 21 bp, Artificial Sequence
  CCHa2_Forward primer
cccgtcaggtgctttacaaaa

SEQ ID NO: 12 - DNA, 20 bp, Artificial Sequence
  CCHa2_Reverse primer
gcgaggtcggttaaaccatg

SEQ ID NO: 13 - DNA, 20 bp, Artificial Sequence
  DH31_Forward primer
cgaaacatcgcatgggtctg

SEQ ID NO: 14 - DNA, 18 bp, Artificial Sequence
  DH31_Reverse primer
tcggtctcggatcgtcgc

SEQ ID NO: 15 - DNA, 20 bp, Artificial Sequence
  TK_Forward primer
tacaagcgtgcagctctctc

SEQ ID NO: 16 - DNA, 20 bp, Artificial Sequence
  TK_Reverse primer
ctccagatcgctcttcttgc

SEQ ID NO: 17 - DNA, 26 bp, Artificial Sequence
  NPF_Forward primer
cataaatctaggaaaaaatgccaaca

SEQ ID NO: 18 - DNA, 19 bp, Artificial Sequence
  NPF_Reverse primer
aaaaccgcgagcaaattct

SEQ ID NO: 19 - DNA, 24 bp, Artificial Sequence
  Dilp3_Forward primer
gtccaggccaccatgaagttgtgc

SEQ ID NO: 20 - DNA, 24 bp, Artificial Sequence
  Dilp3_Reverse primer
ctttccagcagggaacggtcttcg

SEQ ID NO: 21 - DNA, 20 bp, Artificial Sequence
  OrcoB_Forward primer
tccaaaaacaagagccccga

SEQ ID NO: 22 - DNA, 20 bp, Artificial Sequence
  OrcoB_Reverse primer
gtctactctgcgtccgcttt